European Patent Application EP 4 414 455 A1, published August 14, 2024. Title: CONSTRUCT. Applicant: H.U. Group Research Institute G.K. The sequence listing filed with the application follows.

SEQUENCE LISTING (10 sequences)

SEQ ID NO: 1 - DNA, 1164 bp, Homo sapiens
  source 1..1164: mol_type = other DNA
cttcctggcctgggctccgtgccgctctgtttgccaaccgtccagtcccgcctaccagtgccgggcgctccccacccctcccccggctcccccggtgtccgccatggccaaagcctacgaccacctcttcaagttgctgctgatcggggactcgggggtgggcaagacttgtctgatcattcgctttgcagaggacaacttcaacaacacttacatctccaccatcggaattgatttcaagatccgcactgtggatatagaggggaagaagatcaaactacaagtctgggacacggctggccaagagcggttcaagacaataactactgcctactaccgtggagccatgggcattatcctagtatacgacatcacggatgagaaatctttcgagaatattcagaactggatgaaaagcatcaaggagaatgcctcggctggggtggagcgcctcttgctggggaacaaatgtgacatggaggccaagaggaaggtgcagaaggagcaggccgataagttggctcgagagcatggaatccgatttttcgaaactagtgctaaatccagtatgaatgtggatgaggcttttagttccctggcccgggacatcttgctcaagtcaggaggccggagatcaggaaacggcaacaagcctcccagtactgacctgaaaacttgtgacaagaagaacaccaacaagtgctccctgggctgaggaccctttcttgcctccccaccccggaagctgaacctgagggagacaacggcagagggagtgagcaggggagaaatagcagaggggcttggagggtcacataggtagatggtaaagagaatgaggagaaaaaggagaaaagggaaaagcagaaaggaaaaaaaggaagagagaggaagggagaagggagaggaatgaattgaggaagtgaaagaaggcaaggaggtaggaagagagggaggaggaaaggaaggagagatgcctcaggcttcagaccttacctgggttttcagggcaaacataaatgtaaatacactgatttattctgttactagatcaggttttagggtcctgcaaaaggctagctcggcactacactagggaatttgctcctgttctgtcacttgtcatggtctttcttggtattaaaggccaccatttgcacaaat

SEQ ID NO: 2 - DNA, 26 bp, synthetic construct
  misc_feature 1..26: note = Primer
  source 1..26: mol_type = other DNA
atcagcctcgactgtgccttctagtt

SEQ ID NO: 3 - DNA, 25 bp, synthetic construct
  misc_feature 1..25: note = Primer
  source 1..25: mol_type = other DNA
gaaaggacagtgggagtggcacctt

SEQ ID NO: 4 - DNA, 29 bp, synthetic construct
  misc_feature 1..29: note = Primer
  source 1..29: mol_type = other DNA
actttgtcaagctcatttcctggtatgac

SEQ ID NO: 5 - DNA, 30 bp, synthetic construct
  misc_feature 1..30: note = Primer
  source 1..30: mol_type = other DNA
ggtactttattgatggtacatgacaaggtg

SEQ ID NO: 6 - DNA, 393 bp, synthetic construct
  misc_feature 1..393: note = Scramble sequence
  source 1..393: mol_type = other DNA
tgaataaatagaaacaaacatatcatgcaagggttattggccgaaatgtgatggaaagagggtcgattgatcaagatgatcgtggtaaatggaaaagtgacgtacacagctggaagctgtaagtgatcgtagtagcacacagagcagagcgggggatgagcattgtaagtgagccgtgaacctaaggttgaagaaagaggcttgagtaaaaagtagtacagtgagcggattagagaggaggtgagatacgatacgtgcagggggcggaagctacataggacgtagagaggatgcgtacaaagggtattgtgcaacagagtctagggttaaatgaggaattagcctgtgtataagaaagcattgaagtacaaaactgtcgagaaagcaatgcat

SEQ ID NO: 7 - DNA, 20 bp, synthetic construct
  source 1..20: mol_type = other DNA
gactgggtgctcaggtagtg

SEQ ID NO: 8 - DNA, 20 bp, synthetic construct
  source 1..20: mol_type = other DNA
caagatccgccacaacatcg

SEQ ID NO: 9 - DNA, 29 bp, synthetic construct
  source 1..29: mol_type = other DNA
actttgtcaagctcatttcctggtatgac

SEQ ID NO: 10 - DNA, 30 bp, synthetic construct; identical to SEQ ID NO: 5
  source 1..30: mol_type = other DNA